European Patent Specification EP 3 272 860 B1, published August 9, 2023. Title: Pyruvate dehydrogenase variants, a microorganism comprising the same and a method for producing L-amino acid using the same. Applicant: CJ CheilJedang Corporation. The sequence listing filed with the application follows.

SEQUENCE LISTING (33 sequences)

SEQ ID NO: 1 - protein, 922 aa, Corynebacterium glutamicum ATCC13032
MADQAKLGGKPSDDSNFAMIRDGVASYLNDSDPEETNEWMDSLDGLLQESSPERARYLMLRLLERASAKRVSLPPMTSTDYVNTIPTSMEPEFPGDEEMEKRYRRWIRWNAAIMVHRAQRPGIGVGGHISTYAGAAPLYEVGFNHFFRGKDHPGGGDQIFFQGHASPGMYARAFMEGRLSEDDLDGFRQEVSREQGGIPSYPHPHGMKDFWEFPTVSMGLGPMDAIYQARFNRYLENRGIKDTSDQHVWAFLGDGEMDEPESRGLIQQAALNNLDNLTFVVNCNLQRLDGPVRGNTKIIQELESFFRGAGWSVIKVVWGREWDELLEKDQDGALVEIMNNTSDGDYQTFKANDGAYVREHFFGRDPRTAKLVENMTDEEIWKLPRGGHDYRKVYAAYKRALETKDRPTVILAHTIKGYGLGHNFEGRNATHQMKKLTLDDLKLFRDKQGIPITDEQLEKDPYLPPYYHPGEDAPEIKYMKERRAALGGYLPERRENYDPIQVPPLDKLRSVRKGSGKQQIATTMATVRTFKELMRDKGLADRLVPIIPDEARTFGLDSWFPTLKIYNPHGQNYVPVDHDLMLSYREAPEGQILHEGINEAGSVASFIAAGTSYATHGKAMIPLYIFYSMFGFQRTGDSIWAAADQMARGFLLGATAGRTTLTGEGLQHMDGHSPVLASTNEGVETYDPSFAYEIAHLVHRGIDRMYGPGKGEDVIYYITIYNEPTPQPAEPEGLDVEGLHKGIYLYSRGEGTGHEANILASGVGMQWALKAASILEADYGVRANIYSATSWVNLARDGAARNKAQLRNPGADAGEAFVTTQLKQTSGPYVAVSDFSTDLPNQIREWVPGDYTVLGADGFGFSDTRPAARRFFNIDAESIVVAVLNSLAREGKIDVSVAAQAAEKFKLDDPTSVSVDPNAPEE

SEQ ID NO: 2 - DNA, 2769 bp, Corynebacterium glutamicum ATCC13032
atggccgatcaagcaaaacttggtggcaagccctcggatgactctaacttcgcgatgatccgcgatggcgtggcatcttatttgaacgactcagatccggaggagaccaacgagtggatggattcactcgacggattactccaggagtcttctccagaacgtgctcgttacctcatgcttcgtttgcttgagcgtgcatctgcaaagcgcgtatctcttcccccaatgacgtcaaccgactacgtcaacaccattccaacctctatggaacctgaattcccaggcgatgaggaaatggagaagcgttaccgtcgttggattcgctggaacgcagccatcatggttcaccgcgctcagcgaccaggcatcggcgtcggcggacacatttccacttacgcaggcgcagcccctctgtacgaagttggcttcaaccacttcttccgcggcaaggatcacccaggcggcggcgaccagatcttcttccagggccacgcatcaccaggtatgtacgcacgtgcattcatggagggtcgcctttctgaagacgatctcgatggcttccgtcaggaagtttcccgtgagcagggtggcattccgtcctaccctcacccacacggtatgaaggacttctgggagttcccaactgtgtccatgggtcttggcccaatggatgccatttaccaggcacgtttcaaccgctacctcgaaaaccgtggcatcaaggacacctctgaccagcacgtctgggccttccttggcgacggcgaaatggacgagccagaatcacgtggtctcatccagcaggctgcactgaacaacctggacaacctgaccttcgtggttaactgcaacctgcagcgtctcgacggacctgtccgcggtaacaccaagatcatccaggaactcgagtccttcttccgtggcgcaggctggtctgtgatcaaggttgtttggggtcgcgagtgggatgaacttctggagaaggaccaggatggtgcacttgttgagatcatgaacaacacctccgatggtgactaccagaccttcaaggctaacgacggcgcatatgttcgtgagcacttcttcggacgtgacccacgcaccgcaaagctcgttgagaacatgaccgacgaagaaatctggaagcttccacgtggcggccacgattaccgcaaggtttacgcagcctacaagcgagctcttgagaccaaggatcgcccaaccgtcatccttgctcacaccattaagggctacggactcggccacaacttcgaaggccgtaacgcaacccaccagatgaagaagctgacgcttgatgatctgaagttgttccgcgacaagcagggcatcccaatcaccgatgagcagctggagaaggatccttaccttcctccttactaccacccaggtgaagacgctcctgaaatcaagtacatgaaggaacgtcgcgcagcgctcggtggctacctgccagagcgtcgtgagaactacgatccaattcaggttccaccactggataagcttcgctctgtccgtaagggctccggcaagcagcagatcgctaccaccatggcgactgttcgtaccttcaaggaactgatgcgcgataagggcttggctgatcgccttgtcccaatcattcctgatgaggcacgtaccttcggtcttgactcttggttcccaaccttgaagatctacaacccgcacggtcagaactacgtgcctgttgaccacgacctgatgctctcctaccgtgaggcacctgaaggacagatcctgcacgaaggcatcaacgaggctggttccgtggcatcgttcatcgctgcgggtacctcctacgccacccacggcaaggccatgattccgctgtacatcttctactcgatgttcggattccagcgcaccggtgactccatctgggcagcagccgatcagatggcacgtggcttcctcttgggcgctaccgcaggtcgcaccaccctgaccggtgaaggcctccagcacatggatggacactcccctgtcttggcttccaccaacgagggtgtcgagacctacgacccatcctttgcgtacgagatcgcacacctggttcaccgtggcatcgaccgcatgtacggcccaggcaagggtgaagatgttatctactacatcaccatctacaacgagccaaccccacagccagctgagccagaaggactggacgtagaaggcctgcacaagggcatctacctctactcccgcggtgaaggcaccggccatgaggcaaacatcttggcttccggtgttggtatgcagtgggctctcaaggctgcatccatccttgaggctgactacggagttcgtgccaacatttactccgctacttcttgggttaacttggctcgcgatggcgctgctcgtaacaaggcacagctgcgcaacccaggtgcagatgctggcgaggcattcgtaaccacccagctgaagcagacctccggcccatacgttgcagtgtctgacttctccactgatctgccaaaccagatccgtgaatgggtcccaggcgactacaccgttctcggtgcagatggcttcggtttctctgatacccgcccagctgctcgtcgcttcttcaacatcgacgctgagtccattgttgttgcagtgctgaactccctggcacgcgaaggcaagatcgacgtctccgttgctgctcaggctgctgagaagttcaagttggatgatcctacgagtgtttccgtagatccaaacgctcctgaggaataa

SEQ ID NO: 3 - DNA, 18 bp, Artificial Sequence
  Primer 1
tgggaccgggaaaccggg

SEQ ID NO: 4 - DNA, 18 bp, Artificial Sequence
  Primer 2
gatttatctgtcccttga

SEQ ID NO: 5 - DNA, 36 bp, Artificial Sequence
  Primer 3
gcaggtcgactctagatgcgattcgcgtcaaacgtg

SEQ ID NO: 6 - DNA, 30 bp, Artificial Sequence
  Primer 4
gtcccttgaggtgatgtgaatccatccact

SEQ ID NO: 7 - DNA, 30 bp, Artificial Sequence
  Primer 5
agtggatggattcacatcacctcaagggac

SEQ ID NO: 8 - DNA, 36 bp, Artificial Sequence
  Primer 6
ccggggatcctctagacgaagcgccgtgagcaattc

SEQ ID NO: 9 - DNA, 521 bp, Artificial Sequence
  aceE gene fragment comprising 5' end of aceE gene
gcaggtcgactctagatgcgattcgcgtcaaacgtgagagaaacatcacatctcgcgggaaactacccgataattctttgcaaaactttgcaaagcggaatgaacatgcagctagtttccgtagaaatgttctttaaaaaatccacaacaattgccaggaagcacaccgattgatggatacctgaaatcccagtgagcgcaccgctccccttacgtcacagtctgtaaaacaaatcttcggtgttgcgtatccttgttaataacttatgcgttgactcattcgtgcacttcggcgtgtcacaattaggtacgaccaagaatgggaccgggaaaccgggacgtataaacgaaataaaacattccaacaggaggtgtggaaatggccgatcaagcaaaacttggtggcaagccctcggatgactctaacttcgcgatgatccgcgatggcgtggcatcttatttgaacgactcagatccggaggagaccaacgagtggatggattcacatcacctcaagggac

SEQ ID NO: 10 - DNA, 538 bp, Artificial Sequence
  aceE gene fragment comprising 3' end of aceE gene
agtggatggattcacatcacctcaagggacagataaatcccgccgccagacgttagtctggcggcgggattcgtcgtaaagcaagctctttttagccgaggaacgccttgtcagacaatgttgcgcccttgatgttggcgaactcctgcagcaaatcgcgcacagtcaacttcgacttggtagcctgatctgcctggtagacaatctggccttcatgcatcatgatcaggcgattgcccaggcgaattgcctgttccatgttgtgcgtgaccataagcgtagtcagatttccatctgccacgatcttttcggtcaaggtggtcacaagctctgcacgctgtggatcaagcgctgcggtgtgctcatccaacagcatgattttaggttgagtaaaaccagccatcagcagggacaatgcctgacgctgaccgccagagagcaaaccaactttggcagtgagcctgttttccagacccagctcaaggcgctcaagttcctgcttgaattgctcacggcgcttcgtctagaggatccccgg

SEQ ID NO: 11 - DNA, 1029 bp, Artificial Sequence
  Delta aceE
gcaggtcgactctagatgcgattcgcgtcaaacgtgagagaaacatcacatctcgcgggaaactacccgataattctttgcaaaactttgcaaagcggaatgaacatgcagctagtttccgtagaaatgttctttaaaaaatccacaacaattgccaggaagcacaccgattgatggatacctgaaatcccagtgagcgcaccgctccccttacgtcacagtctgtaaaacaaatcttcggtgttgcgtatccttgttaataacttatgcgttgactcattcgtgcacttcggcgtgtcacaattaggtacgaccaagaatgggaccgggaaaccgggacgtataaacgaaataaaacattccaacaggaggtgtggaaatggccgatcaagcaaaacttggtggcaagccctcggatgactctaacttcgcgatgatccgcgatggcgtggcatcttatttgaacgactcagatccggaggagaccaacgagtggatggattcacatcacctcaagggacagataaatcccgccgccagacgttagtctggcggcgggattcgtcgtaaagcaagctctttttagccgaggaacgccttgtcagacaatgttgcgcccttgatgttggcgaactcctgcagcaaatcgcgcacagtcaacttcgacttggtagcctgatctgcctggtagacaatctggccttcatgcatcatgatcaggcgattgcccaggcgaattgcctgttccatgttgtgcgtgaccataagcgtagtcagatttccatctgccacgatcttttcggtcaaggtggtcacaagctctgcacgctgtggatcaagcgctgcggtgtgctcatccaacagcatgattttaggttgagtaaaaccagccatcagcagggacaatgcctgacgctgaccgccagagagcaaaccaactttggcagtgagcctgttttccagacccagctcaaggcgctcaagttcctgcttgaattgctcacggcgcttcgtctagaggatccccgg

SEQ ID NO: 12 - DNA, 26 bp, Artificial Sequence
  Primer 9
aatctagatgggaccgggaaaccggg

SEQ ID NO: 13 - DNA, 26 bp, Artificial Sequence
  Primer 10
aatctagagatttatctgtcccttga

SEQ ID NO: 14 - protein, 922 aa, Artificial Sequence
  E1p(Q432E)
MADQAKLGGKPSDDSNFAMIRDGVASYLNDSDPEETNEWMDSLDGLLQESSPERARYLMLRLLERASAKRVSLPPMTSTDYVNTIPTSMEPEFPGDEEMEKRYRRWIRWNAAIMVHRAQRPGIGVGGHISTYAGAAPLYEVGFNHFFRGKDHPGGGDQIFFQGHASPGMYARAFMEGRLSEDDLDGFRQEVSREQGGIPSYPHPHGMKDFWEFPTVSMGLGPMDAIYQARFNRYLENRGIKDTSDQHVWAFLGDGEMDEPESRGLIQQAALNNLDNLTFVVNCNLQRLDGPVRGNTKIIQELESFFRGAGWSVIKVVWGREWDELLEKDQDGALVEIMNNTSDGDYQTFKANDGAYVREHFFGRDPRTAKLVENMTDEEIWKLPRGGHDYRKVYAAYKRALETKDRPTVILAHTIKGYGLGHNFEGRNATHEMKKLTLDDLKLFRDKQGIPITDEQLEKDPYLPPYYHPGEDAPEIKYMKERRAALGGYLPERRENYDPIQVPPLDKLRSVRKGSGKQQIATTMATVRTFKELMRDKGLADRLVPIIPDEARTFGLDSWFPTLKIYNPHGQNYVPVDHDLMLSYREAPEGQILHEGINEAGSVASFIAAGTSYATHGKAMIPLYIFYSMFGFQRTGDSIWAAADQMARGFLLGATAGRTTLTGEGLQHMDGHSPVLASTNEGVETYDPSFAYEIAHLVHRGIDRMYGPGKGEDVIYYITIYNEPTPQPAEPEGLDVEGLHKGIYLYSRGEGTGHEANILASGVGMQWALKAASILEADYGVRANIYSATSWVNLARDGAARNKAQLRNPGADAGEAFVTTQLKQTSGPYVAVSDFSTDLPNQIREWVPGDYTVLGADGFGFSDTRPAARRFFNIDAESIVVAVLNSLAREGKIDVSVAAQAAEKFKLDDPTSVSVDPNAPEE

SEQ ID NO: 15 - protein, 922 aa, Artificial Sequence
  E1p(E190V)
MADQAKLGGKPSDDSNFAMIRDGVASYLNDSDPEETNEWMDSLDGLLQESSPERARYLMLRLLERASAKRVSLPPMTSTDYVNTIPTSMEPEFPGDEEMEKRYRRWIRWNAAIMVHRAQRPGIGVGGHISTYAGAAPLYEVGFNHFFRGKDHPGGGDQIFFQGHASPGMYARAFMEGRLSEDDLDGFRQVVSREQGGIPSYPHPHGMKDFWEFPTVSMGLGPMDAIYQARFNRYLENRGIKDTSDQHVWAFLGDGEMDEPESRGLIQQAALNNLDNLTFVVNCNLQRLDGPVRGNTKIIQELESFFRGAGWSVIKVVWGREWDELLEKDQDGALVEIMNNTSDGDYQTFKANDGAYVREHFFGRDPRTAKLVENMTDEEIWKLPRGGHDYRKVYAAYKRALETKDRPTVILAHTIKGYGLGHNFEGRNATHQMKKLTLDDLKLFRDKQGIPITDEQLEKDPYLPPYYHPGEDAPEIKYMKERRAALGGYLPERRENYDPIQVPPLDKLRSVRKGSGKQQIATTMATVRTFKELMRDKGLADRLVPIIPDEARTFGLDSWFPTLKIYNPHGQNYVPVDHDLMLSYREAPEGQILHEGINEAGSVASFIAAGTSYATHGKAMIPLYIFYSMFGFQRTGDSIWAAADQMARGFLLGATAGRTTLTGEGLQHMDGHSPVLASTNEGVETYDPSFAYEIAHLVHRGIDRMYGPGKGEDVIYYITIYNEPTPQPAEPEGLDVEGLHKGIYLYSRGEGTGHEANILASGVGMQWALKAASILEADYGVRANIYSATSWVNLARDGAARNKAQLRNPGADAGEAFVTTQLKQTSGPYVAVSDFSTDLPNQIREWVPGDYTVLGADGFGFSDTRPAARRFFNIDAESIVVAVLNSLAREGKIDVSVAAQAAEKFKLDDPTSVSVDPNAPEE

SEQ ID NO: 16 - protein, 922 aa, Artificial Sequence
  E1p(L438P)
MADQAKLGGKPSDDSNFAMIRDGVASYLNDSDPEETNEWMDSLDGLLQESSPERARYLMLRLLERASAKRVSLPPMTSTDYVNTIPTSMEPEFPGDEEMEKRYRRWIRWNAAIMVHRAQRPGIGVGGHISTYAGAAPLYEVGFNHFFRGKDHPGGGDQIFFQGHASPGMYARAFMEGRLSEDDLDGFRQEVSREQGGIPSYPHPHGMKDFWEFPTVSMGLGPMDAIYQARFNRYLENRGIKDTSDQHVWAFLGDGEMDEPESRGLIQQAALNNLDNLTFVVNCNLQRLDGPVRGNTKIIQELESFFRGAGWSVIKVVWGREWDELLEKDQDGALVEIMNNTSDGDYQTFKANDGAYVREHFFGRDPRTAKLVENMTDEEIWKLPRGGHDYRKVYAAYKRALETKDRPTVILAHTIKGYGLGHNFEGRNATHQMKKLTPDDLKLFRDKQGIPITDEQLEKDPYLPPYYHPGEDAPEIKYMKERRAALGGYLPERRENYDPIQVPPLDKLRSVRKGSGKQQIATTMATVRTFKELMRDKGLADRLVPIIPDEARTFGLDSWFPTLKIYNPHGQNYVPVDHDLMLSYREAPEGQILHEGINEAGSVASFIAAGTSYATHGKAMIPLYIFYSMFGFQRTGDSIWAAADQMARGFLLGATAGRTTLTGEGLQHMDGHSPVLASTNEGVETYDPSFAYEIAHLVHRGIDRMYGPGKGEDVIYYITIYNEPTPQPAEPEGLDVEGLHKGIYLYSRGEGTGHEANILASGVGMQWALKAASILEADYGVRANIYSATSWVNLARDGAARNKAQLRNPGADAGEAFVTTQLKQTSGPYVAVSDFSTDLPNQIREWVPGDYTVLGADGFGFSDTRPAARRFFNIDAESIVVAVLNSLAREGKIDVSVAAQAAEKFKLDDPTSVSVDPNAPEE

SEQ ID NO: 17 - protein, 922 aa, Artificial Sequence
  E1p(Q195H)
MADQAKLGGKPSDDSNFAMIRDGVASYLNDSDPEETNEWMDSLDGLLQESSPERARYLMLRLLERASAKRVSLPPMTSTDYVNTIPTSMEPEFPGDEEMEKRYRRWIRWNAAIMVHRAQRPGIGVGGHISTYAGAAPLYEVGFNHFFRGKDHPGGGDQIFFQGHASPGMYARAFMEGRLSEDDLDGFRQEVSREHGGIPSYPHPHGMKDFWEFPTVSMGLGPMDAIYQARFNRYLENRGIKDTSDQHVWAFLGDGEMDEPESRGLIQQAALNNLDNLTFVVNCNLQRLDGPVRGNTKIIQELESFFRGAGWSVIKVVWGREWDELLEKDQDGALVEIMNNTSDGDYQTFKANDGAYVREHFFGRDPRTAKLVENMTDEEIWKLPRGGHDYRKVYAAYKRALETKDRPTVILAHTIKGYGLGHNFEGRNATHQMKKLTLDDLKLFRDKQGIPITDEQLEKDPYLPPYYHPGEDAPEIKYMKERRAALGGYLPERRENYDPIQVPPLDKLRSVRKGSGKQQIATTMATVRTFKELMRDKGLADRLVPIIPDEARTFGLDSWFPTLKIYNPHGQNYVPVDHDLMLSYREAPEGQILHEGINEAGSVASFIAAGTSYATHGKAMIPLYIFYSMFGFQRTGDSIWAAADQMARGFLLGATAGRTTLTGEGLQHMDGHSPVLASTNEGVETYDPSFAYEIAHLVHRGIDRMYGPGKGEDVIYYITIYNEPTPQPAEPEGLDVEGLHKGIYLYSRGEGTGHEANILASGVGMQWALKAASILEADYGVRANIYSATSWVNLARDGAARNKAQLRNPGADAGEAFVTTQLKQTSGPYVAVSDFSTDLPNQIREWVPGDYTVLGADGFGFSDTRPAARRFFNIDAESIVVAVLNSLAREGKIDVSVAAQAAEKFKLDDPTSVSVDPNAPEE

SEQ ID NO: 18 - protein, 922 aa, Artificial Sequence
  E1p(P199S)
MADQAKLGGKPSDDSNFAMIRDGVASYLNDSDPEETNEWMDSLDGLLQESSPERARYLMLRLLERASAKRVSLPPMTSTDYVNTIPTSMEPEFPGDEEMEKRYRRWIRWNAAIMVHRAQRPGIGVGGHISTYAGAAPLYEVGFNHFFRGKDHPGGGDQIFFQGHASPGMYARAFMEGRLSEDDLDGFRQEVSREQGGISSYPHPHGMKDFWEFPTVSMGLGPMDAIYQARFNRYLENRGIKDTSDQHVWAFLGDGEMDEPESRGLIQQAALNNLDNLTFVVNCNLQRLDGPVRGNTKIIQELESFFRGAGWSVIKVVWGREWDELLEKDQDGALVEIMNNTSDGDYQTFKANDGAYVREHFFGRDPRTAKLVENMTDEEIWKLPRGGHDYRKVYAAYKRALETKDRPTVILAHTIKGYGLGHNFEGRNATHQMKKLTLDDLKLFRDKQGIPITDEQLEKDPYLPPYYHPGEDAPEIKYMKERRAALGGYLPERRENYDPIQVPPLDKLRSVRKGSGKQQIATTMATVRTFKELMRDKGLADRLVPIIPDEARTFGLDSWFPTLKIYNPHGQNYVPVDHDLMLSYREAPEGQILHEGINEAGSVASFIAAGTSYATHGKAMIPLYIFYSMFGFQRTGDSIWAAADQMARGFLLGATAGRTTLTGEGLQHMDGHSPVLASTNEGVETYDPSFAYEIAHLVHRGIDRMYGPGKGEDVIYYITIYNEPTPQPAEPEGLDVEGLHKGIYLYSRGEGTGHEANILASGVGMQWALKAASILEADYGVRANIYSATSWVNLARDGAARNKAQLRNPGADAGEAFVTTQLKQTSGPYVAVSDFSTDLPNQIREWVPGDYTVLGADGFGFSDTRPAARRFFNIDAESIVVAVLNSLAREGKIDVSVAAQAAEKFKLDDPTSVSVDPNAPEE

SEQ ID NO: 19 - protein, 922 aa, Artificial Sequence
  E1p(K435A)
MADQAKLGGKPSDDSNFAMIRDGVASYLNDSDPEETNEWMDSLDGLLQESSPERARYLMLRLLERASAKRVSLPPMTSTDYVNTIPTSMEPEFPGDEEMEKRYRRWIRWNAAIMVHRAQRPGIGVGGHISTYAGAAPLYEVGFNHFFRGKDHPGGGDQIFFQGHASPGMYARAFMEGRLSEDDLDGFRQEVSREQGGIPSYPHPHGMKDFWEFPTVSMGLGPMDAIYQARFNRYLENRGIKDTSDQHVWAFLGDGEMDEPESRGLIQQAALNNLDNLTFVVNCNLQRLDGPVRGNTKIIQELESFFRGAGWSVIKVVWGREWDELLEKDQDGALVEIMNNTSDGDYQTFKANDGAYVREHFFGRDPRTAKLVENMTDEEIWKLPRGGHDYRKVYAAYKRALETKDRPTVILAHTIKGYGLGHNFEGRNATHQMKALTLDDLKLFRDKQGIPITDEQLEKDPYLPPYYHPGEDAPEIKYMKERRAALGGYLPERRENYDPIQVPPLDKLRSVRKGSGKQQIATTMATVRTFKELMRDKGLADRLVPIIPDEARTFGLDSWFPTLKIYNPHGQNYVPVDHDLMLSYREAPEGQILHEGINEAGSVASFIAAGTSYATHGKAMIPLYIFYSMFGFQRTGDSIWAAADQMARGFLLGATAGRTTLTGEGLQHMDGHSPVLASTNEGVETYDPSFAYEIAHLVHRGIDRMYGPGKGEDVIYYITIYNEPTPQPAEPEGLDVEGLHKGIYLYSRGEGTGHEANILASGVGMQWALKAASILEADYGVRANIYSATSWVNLARDGAARNKAQLRNPGADAGEAFVTTQLKQTSGPYVAVSDFSTDLPNQIREWVPGDYTVLGADGFGFSDTRPAARRFFNIDAESIVVAVLNSLAREGKIDVSVAAQAAEKFKLDDPTSVSVDPNAPEE

SEQ ID NO: 20 - protein, 922 aa, Artificial Sequence
  E1p(Q432A)
MADQAKLGGKPSDDSNFAMIRDGVASYLNDSDPEETNEWMDSLDGLLQESSPERARYLMLRLLERASAKRVSLPPMTSTDYVNTIPTSMEPEFPGDEEMEKRYRRWIRWNAAIMVHRAQRPGIGVGGHISTYAGAAPLYEVGFNHFFRGKDHPGGGDQIFFQGHASPGMYARAFMEGRLSEDDLDGFRQEVSREQGGIPSYPHPHGMKDFWEFPTVSMGLGPMDAIYQARFNRYLENRGIKDTSDQHVWAFLGDGEMDEPESRGLIQQAALNNLDNLTFVVNCNLQRLDGPVRGNTKIIQELESFFRGAGWSVIKVVWGREWDELLEKDQDGALVEIMNNTSDGDYQTFKANDGAYVREHFFGRDPRTAKLVENMTDEEIWKLPRGGHDYRKVYAAYKRALETKDRPTVILAHTIKGYGLGHNFEGRNATHAMKKLTLDDLKLFRDKQGIPITDEQLEKDPYLPPYYHPGEDAPEIKYMKERRAALGGYLPERRENYDPIQVPPLDKLRSVRKGSGKQQIATTMATVRTFKELMRDKGLADRLVPIIPDEARTFGLDSWFPTLKIYNPHGQNYVPVDHDLMLSYREAPEGQILHEGINEAGSVASFIAAGTSYATHGKAMIPLYIFYSMFGFQRTGDSIWAAADQMARGFLLGATAGRTTLTGEGLQHMDGHSPVLASTNEGVETYDPSFAYEIAHLVHRGIDRMYGPGKGEDVIYYITIYNEPTPQPAEPEGLDVEGLHKGIYLYSRGEGTGHEANILASGVGMQWALKAASILEADYGVRANIYSATSWVNLARDGAARNKAQLRNPGADAGEAFVTTQLKQTSGPYVAVSDFSTDLPNQIREWVPGDYTVLGADGFGFSDTRPAARRFFNIDAESIVVAVLNSLAREGKIDVSVAAQAAEKFKLDDPTSVSVDPNAPEE

SEQ ID NO: 21 - protein, 922 aa, Artificial Sequence
  E1p(Y418H)
MADQAKLGGKPSDDSNFAMIRDGVASYLNDSDPEETNEWMDSLDGLLQESSPERARYLMLRLLERASAKRVSLPPMTSTDYVNTIPTSMEPEFPGDEEMEKRYRRWIRWNAAIMVHRAQRPGIGVGGHISTYAGAAPLYEVGFNHFFRGKDHPGGGDQIFFQGHASPGMYARAFMEGRLSEDDLDGFRQEVSREQGGIPSYPHPHGMKDFWEFPTVSMGLGPMDAIYQARFNRYLENRGIKDTSDQHVWAFLGDGEMDEPESRGLIQQAALNNLDNLTFVVNCNLQRLDGPVRGNTKIIQELESFFRGAGWSVIKVVWGREWDELLEKDQDGALVEIMNNTSDGDYQTFKANDGAYVREHFFGRDPRTAKLVENMTDEEIWKLPRGGHDYRKVYAAYKRALETKDRPTVILAHTIKGHGLGHNFEGRNATHQMKKLTLDDLKLFRDKQGIPITDEQLEKDPYLPPYYHPGEDAPEIKYMKERRAALGGYLPERRENYDPIQVPPLDKLRSVRKGSGKQQIATTMATVRTFKELMRDKGLADRLVPIIPDEARTFGLDSWFPTLKIYNPHGQNYVPVDHDLMLSYREAPEGQILHEGINEAGSVASFIAAGTSYATHGKAMIPLYIFYSMFGFQRTGDSIWAAADQMARGFLLGATAGRTTLTGEGLQHMDGHSPVLASTNEGVETYDPSFAYEIAHLVHRGIDRMYGPGKGEDVIYYITIYNEPTPQPAEPEGLDVEGLHKGIYLYSRGEGTGHEANILASGVGMQWALKAASILEADYGVRANIYSATSWVNLARDGAARNKAQLRNPGADAGEAFVTTQLKQTSGPYVAVSDFSTDLPNQIREWVPGDYTVLGADGFGFSDTRPAARRFFNIDAESIVVAVLNSLAREGKIDVSVAAQAAEKFKLDDPTSVSVDPNAPEE

SEQ ID NO: 22 - protein, 922 aa, Artificial Sequence
  E1p(Y201A)
MADQAKLGGKPSDDSNFAMIRDGVASYLNDSDPEETNEWMDSLDGLLQESSPERARYLMLRLLERASAKRVSLPPMTSTDYVNTIPTSMEPEFPGDEEMEKRYRRWIRWNAAIMVHRAQRPGIGVGGHISTYAGAAPLYEVGFNHFFRGKDHPGGGDQIFFQGHASPGMYARAFMEGRLSEDDLDGFRQEVSREQGGIPSAPHPHGMKDFWEFPTVSMGLGPMDAIYQARFNRYLENRGIKDTSDQHVWAFLGDGEMDEPESRGLIQQAALNNLDNLTFVVNCNLQRLDGPVRGNTKIIQELESFFRGAGWSVIKVVWGREWDELLEKDQDGALVEIMNNTSDGDYQTFKANDGAYVREHFFGRDPRTAKLVENMTDEEIWKLPRGGHDYRKVYAAYKRALETKDRPTVILAHTIKGYGLGHNFEGRNATHQMKKLTLDDLKLFRDKQGIPITDEQLEKDPYLPPYYHPGEDAPEIKYMKERRAALGGYLPERRENYDPIQVPPLDKLRSVRKGSGKQQIATTMATVRTFKELMRDKGLADRLVPIIPDEARTFGLDSWFPTLKIYNPHGQNYVPVDHDLMLSYREAPEGQILHEGINEAGSVASFIAAGTSYATHGKAMIPLYIFYSMFGFQRTGDSIWAAADQMARGFLLGATAGRTTLTGEGLQHMDGHSPVLASTNEGVETYDPSFAYEIAHLVHRGIDRMYGPGKGEDVIYYITIYNEPTPQPAEPEGLDVEGLHKGIYLYSRGEGTGHEANILASGVGMQWALKAASILEADYGVRANIYSATSWVNLARDGAARNKAQLRNPGADAGEAFVTTQLKQTSGPYVAVSDFSTDLPNQIREWVPGDYTVLGADGFGFSDTRPAARRFFNIDAESIVVAVLNSLAREGKIDVSVAAQAAEKFKLDDPTSVSVDPNAPEE

SEQ ID NO: 23 - protein, 922 aa, Artificial Sequence
  E1p(N428A)
MADQAKLGGKPSDDSNFAMIRDGVASYLNDSDPEETNEWMDSLDGLLQESSPERARYLMLRLLERASAKRVSLPPMTSTDYVNTIPTSMEPEFPGDEEMEKRYRRWIRWNAAIMVHRAQRPGIGVGGHISTYAGAAPLYEVGFNHFFRGKDHPGGGDQIFFQGHASPGMYARAFMEGRLSEDDLDGFRQEVSREQGGIPSYPHPHGMKDFWEFPTVSMGLGPMDAIYQARFNRYLENRGIKDTSDQHVWAFLGDGEMDEPESRGLIQQAALNNLDNLTFVVNCNLQRLDGPVRGNTKIIQELESFFRGAGWSVIKVVWGREWDELLEKDQDGALVEIMNNTSDGDYQTFKANDGAYVREHFFGRDPRTAKLVENMTDEEIWKLPRGGHDYRKVYAAYKRALETKDRPTVILAHTIKGYGLGHNFEGRAATHQMKKLTLDDLKLFRDKQGIPITDEQLEKDPYLPPYYHPGEDAPEIKYMKERRAALGGYLPERRENYDPIQVPPLDKLRSVRKGSGKQQIATTMATVRTFKELMRDKGLADRLVPIIPDEARTFGLDSWFPTLKIYNPHGQNYVPVDHDLMLSYREAPEGQILHEGINEAGSVASFIAAGTSYATHGKAMIPLYIFYSMFGFQRTGDSIWAAADQMARGFLLGATAGRTTLTGEGLQHMDGHSPVLASTNEGVETYDPSFAYEIAHLVHRGIDRMYGPGKGEDVIYYITIYNEPTPQPAEPEGLDVEGLHKGIYLYSRGEGTGHEANILASGVGMQWALKAASILEADYGVRANIYSATSWVNLARDGAARNKAQLRNPGADAGEAFVTTQLKQTSGPYVAVSDFSTDLPNQIREWVPGDYTVLGADGFGFSDTRPAARRFFNIDAESIVVAVLNSLAREGKIDVSVAAQAAEKFKLDDPTSVSVDPNAPEE

SEQ ID NO: 24 - protein, 922 aa, Artificial Sequence
  E190V, Q195H
MADQAKLGGKPSDDSNFAMIRDGVASYLNDSDPEETNEWMDSLDGLLQESSPERARYLMLRLLERASAKRVSLPPMTSTDYVNTIPTSMEPEFPGDEEMEKRYRRWIRWNAAIMVHRAQRPGIGVGGHISTYAGAAPLYEVGFNHFFRGKDHPGGGDQIFFQGHASPGMYARAFMEGRLSEDDLDGFRQVVSREHGGIPSYPHPHGMKDFWEFPTVSMGLGPMDAIYQARFNRYLENRGIKDTSDQHVWAFLGDGEMDEPESRGLIQQAALNNLDNLTFVVNCNLQRLDGPVRGNTKIIQELESFFRGAGWSVIKVVWGREWDELLEKDQDGALVEIMNNTSDGDYQTFKANDGAYVREHFFGRDPRTAKLVENMTDEEIWKLPRGGHDYRKVYAAYKRALETKDRPTVILAHTIKGYGLGHNFEGRNATHQMKKLTLDDLKLFRDKQGIPITDEQLEKDPYLPPYYHPGEDAPEIKYMKERRAALGGYLPERRENYDPIQVPPLDKLRSVRKGSGKQQIATTMATVRTFKELMRDKGLADRLVPIIPDEARTFGLDSWFPTLKIYNPHGQNYVPVDHDLMLSYREAPEGQILHEGINEAGSVASFIAAGTSYATHGKAMIPLYIFYSMFGFQRTGDSIWAAADQMARGFLLGATAGRTTLTGEGLQHMDGHSPVLASTNEGVETYDPSFAYEIAHLVHRGIDRMYGPGKGEDVIYYITIYNEPTPQPAEPEGLDVEGLHKGIYLYSRGEGTGHEANILASGVGMQWALKAASILEADYGVRANIYSATSWVNLARDGAARNKAQLRNPGADAGEAFVTTQLKQTSGPYVAVSDFSTDLPNQIREWVPGDYTVLGADGFGFSDTRPAARRFFNIDAESIVVAVLNSLAREGKIDVSVAAQAAEKFKLDDPTSVSVDPNAPEE

SEQ ID NO: 25 - protein, 922 aa, Artificial Sequence
  E190V, P199S
MADQAKLGGKPSDDSNFAMIRDGVASYLNDSDPEETNEWMDSLDGLLQESSPERARYLMLRLLERASAKRVSLPPMTSTDYVNTIPTSMEPEFPGDEEMEKRYRRWIRWNAAIMVHRAQRPGIGVGGHISTYAGAAPLYEVGFNHFFRGKDHPGGGDQIFFQGHASPGMYARAFMEGRLSEDDLDGFRQVVSREQGGISSYPHPHGMKDFWEFPTVSMGLGPMDAIYQARFNRYLENRGIKDTSDQHVWAFLGDGEMDEPESRGLIQQAALNNLDNLTFVVNCNLQRLDGPVRGNTKIIQELESFFRGAGWSVIKVVWGREWDELLEKDQDGALVEIMNNTSDGDYQTFKANDGAYVREHFFGRDPRTAKLVENMTDEEIWKLPRGGHDYRKVYAAYKRALETKDRPTVILAHTIKGYGLGHNFEGRNATHQMKKLTLDDLKLFRDKQGIPITDEQLEKDPYLPPYYHPGEDAPEIKYMKERRAALGGYLPERRENYDPIQVPPLDKLRSVRKGSGKQQIATTMATVRTFKELMRDKGLADRLVPIIPDEARTFGLDSWFPTLKIYNPHGQNYVPVDHDLMLSYREAPEGQILHEGINEAGSVASFIAAGTSYATHGKAMIPLYIFYSMFGFQRTGDSIWAAADQMARGFLLGATAGRTTLTGEGLQHMDGHSPVLASTNEGVETYDPSFAYEIAHLVHRGIDRMYGPGKGEDVIYYITIYNEPTPQPAEPEGLDVEGLHKGIYLYSRGEGTGHEANILASGVGMQWALKAASILEADYGVRANIYSATSWVNLARDGAARNKAQLRNPGADAGEAFVTTQLKQTSGPYVAVSDFSTDLPNQIREWVPGDYTVLGADGFGFSDTRPAARRFFNIDAESIVVAVLNSLAREGKIDVSVAAQAAEKFKLDDPTSVSVDPNAPEE

SEQ ID NO: 26 - protein, 922 aa, Artificial Sequence
  Q195H, P199S
MADQAKLGGKPSDDSNFAMIRDGVASYLNDSDPEETNEWMDSLDGLLQESSPERARYLMLRLLERASAKRVSLPPMTSTDYVNTIPTSMEPEFPGDEEMEKRYRRWIRWNAAIMVHRAQRPGIGVGGHISTYAGAAPLYEVGFNHFFRGKDHPGGGDQIFFQGHASPGMYARAFMEGRLSEDDLDGFRQEVSREHGGISSYPHPHGMKDFWEFPTVSMGLGPMDAIYQARFNRYLENRGIKDTSDQHVWAFLGDGEMDEPESRGLIQQAALNNLDNLTFVVNCNLQRLDGPVRGNTKIIQELESFFRGAGWSVIKVVWGREWDELLEKDQDGALVEIMNNTSDGDYQTFKANDGAYVREHFFGRDPRTAKLVENMTDEEIWKLPRGGHDYRKVYAAYKRALETKDRPTVILAHTIKGYGLGHNFEGRNATHQMKKLTLDDLKLFRDKQGIPITDEQLEKDPYLPPYYHPGEDAPEIKYMKERRAALGGYLPERRENYDPIQVPPLDKLRSVRKGSGKQQIATTMATVRTFKELMRDKGLADRLVPIIPDEARTFGLDSWFPTLKIYNPHGQNYVPVDHDLMLSYREAPEGQILHEGINEAGSVASFIAAGTSYATHGKAMIPLYIFYSMFGFQRTGDSIWAAADQMARGFLLGATAGRTTLTGEGLQHMDGHSPVLASTNEGVETYDPSFAYEIAHLVHRGIDRMYGPGKGEDVIYYITIYNEPTPQPAEPEGLDVEGLHKGIYLYSRGEGTGHEANILASGVGMQWALKAASILEADYGVRANIYSATSWVNLARDGAARNKAQLRNPGADAGEAFVTTQLKQTSGPYVAVSDFSTDLPNQIREWVPGDYTVLGADGFGFSDTRPAARRFFNIDAESIVVAVLNSLAREGKIDVSVAAQAAEKFKLDDPTSVSVDPNAPEE

SEQ ID NO: 27 - protein, 922 aa, Artificial Sequence
  E190V, Y201A
MADQAKLGGKPSDDSNFAMIRDGVASYLNDSDPEETNEWMDSLDGLLQESSPERARYLMLRLLERASAKRVSLPPMTSTDYVNTIPTSMEPEFPGDEEMEKRYRRWIRWNAAIMVHRAQRPGIGVGGHISTYAGAAPLYEVGFNHFFRGKDHPGGGDQIFFQGHASPGMYARAFMEGRLSEDDLDGFRQVVSREQGGIPSAPHPHGMKDFWEFPTVSMGLGPMDAIYQARFNRYLENRGIKDTSDQHVWAFLGDGEMDEPESRGLIQQAALNNLDNLTFVVNCNLQRLDGPVRGNTKIIQELESFFRGAGWSVIKVVWGREWDELLEKDQDGALVEIMNNTSDGDYQTFKANDGAYVREHFFGRDPRTAKLVENMTDEEIWKLPRGGHDYRKVYAAYKRALETKDRPTVILAHTIKGYGLGHNFEGRNATHQMKKLTLDDLKLFRDKQGIPITDEQLEKDPYLPPYYHPGEDAPEIKYMKERRAALGGYLPERRENYDPIQVPPLDKLRSVRKGSGKQQIATTMATVRTFKELMRDKGLADRLVPIIPDEARTFGLDSWFPTLKIYNPHGQNYVPVDHDLMLSYREAPEGQILHEGINEAGSVASFIAAGTSYATHGKAMIPLYIFYSMFGFQRTGDSIWAAADQMARGFLLGATAGRTTLTGEGLQHMDGHSPVLASTNEGVETYDPSFAYEIAHLVHRGIDRMYGPGKGEDVIYYITIYNEPTPQPAEPEGLDVEGLHKGIYLYSRGEGTGHEANILASGVGMQWALKAASILEADYGVRANIYSATSWVNLARDGAARNKAQLRNPGADAGEAFVTTQLKQTSGPYVAVSDFSTDLPNQIREWVPGDYTVLGADGFGFSDTRPAARRFFNIDAESIVVAVLNSLAREGKIDVSVAAQAAEKFKLDDPTSVSVDPNAPEE

SEQ ID NO: 28 - protein, 922 aa, Artificial Sequence
  Q195H, Y201A
MADQAKLGGKPSDDSNFAMIRDGVASYLNDSDPEETNEWMDSLDGLLQESSPERARYLMLRLLERASAKRVSLPPMTSTDYVNTIPTSMEPEFPGDEEMEKRYRRWIRWNAAIMVHRAQRPGIGVGGHISTYAGAAPLYEVGFNHFFRGKDHPGGGDQIFFQGHASPGMYARAFMEGRLSEDDLDGFRQEVSREHGGIPSAPHPHGMKDFWEFPTVSMGLGPMDAIYQARFNRYLENRGIKDTSDQHVWAFLGDGEMDEPESRGLIQQAALNNLDNLTFVVNCNLQRLDGPVRGNTKIIQELESFFRGAGWSVIKVVWGREWDELLEKDQDGALVEIMNNTSDGDYQTFKANDGAYVREHFFGRDPRTAKLVENMTDEEIWKLPRGGHDYRKVYAAYKRALETKDRPTVILAHTIKGYGLGHNFEGRNATHQMKKLTLDDLKLFRDKQGIPITDEQLEKDPYLPPYYHPGEDAPEIKYMKERRAALGGYLPERRENYDPIQVPPLDKLRSVRKGSGKQQIATTMATVRTFKELMRDKGLADRLVPIIPDEARTFGLDSWFPTLKIYNPHGQNYVPVDHDLMLSYREAPEGQILHEGINEAGSVASFIAAGTSYATHGKAMIPLYIFYSMFGFQRTGDSIWAAADQMARGFLLGATAGRTTLTGEGLQHMDGHSPVLASTNEGVETYDPSFAYEIAHLVHRGIDRMYGPGKGEDVIYYITIYNEPTPQPAEPEGLDVEGLHKGIYLYSRGEGTGHEANILASGVGMQWALKAASILEADYGVRANIYSATSWVNLARDGAARNKAQLRNPGADAGEAFVTTQLKQTSGPYVAVSDFSTDLPNQIREWVPGDYTVLGADGFGFSDTRPAARRFFNIDAESIVVAVLNSLAREGKIDVSVAAQAAEKFKLDDPTSVSVDPNAPEE

SEQ ID NO: 29 - protein, 922 aa, Artificial Sequence
  P199S, Y201A
MADQAKLGGKPSDDSNFAMIRDGVASYLNDSDPEETNEWMDSLDGLLQESSPERARYLMLRLLERASAKRVSLPPMTSTDYVNTIPTSMEPEFPGDEEMEKRYRRWIRWNAAIMVHRAQRPGIGVGGHISTYAGAAPLYEVGFNHFFRGKDHPGGGDQIFFQGHASPGMYARAFMEGRLSEDDLDGFRQEVSREQGGISSAPHPHGMKDFWEFPTVSMGLGPMDAIYQARFNRYLENRGIKDTSDQHVWAFLGDGEMDEPESRGLIQQAALNNLDNLTFVVNCNLQRLDGPVRGNTKIIQELESFFRGAGWSVIKVVWGREWDELLEKDQDGALVEIMNNTSDGDYQTFKANDGAYVREHFFGRDPRTAKLVENMTDEEIWKLPRGGHDYRKVYAAYKRALETKDRPTVILAHTIKGYGLGHNFEGRNATHQMKKLTLDDLKLFRDKQGIPITDEQLEKDPYLPPYYHPGEDAPEIKYMKERRAALGGYLPERRENYDPIQVPPLDKLRSVRKGSGKQQIATTMATVRTFKELMRDKGLADRLVPIIPDEARTFGLDSWFPTLKIYNPHGQNYVPVDHDLMLSYREAPEGQILHEGINEAGSVASFIAAGTSYATHGKAMIPLYIFYSMFGFQRTGDSIWAAADQMARGFLLGATAGRTTLTGEGLQHMDGHSPVLASTNEGVETYDPSFAYEIAHLVHRGIDRMYGPGKGEDVIYYITIYNEPTPQPAEPEGLDVEGLHKGIYLYSRGEGTGHEANILASGVGMQWALKAASILEADYGVRANIYSATSWVNLARDGAARNKAQLRNPGADAGEAFVTTQLKQTSGPYVAVSDFSTDLPNQIREWVPGDYTVLGADGFGFSDTRPAARRFFNIDAESIVVAVLNSLAREGKIDVSVAAQAAEKFKLDDPTSVSVDPNAPEE

SEQ ID NO: 30 - protein, 922 aa, Artificial Sequence
  N428A, Q432E
MADQAKLGGKPSDDSNFAMIRDGVASYLNDSDPEETNEWMDSLDGLLQESSPERARYLMLRLLERASAKRVSLPPMTSTDYVNTIPTSMEPEFPGDEEMEKRYRRWIRWNAAIMVHRAQRPGIGVGGHISTYAGAAPLYEVGFNHFFRGKDHPGGGDQIFFQGHASPGMYARAFMEGRLSEDDLDGFRQEVSREQGGIPSYPHPHGMKDFWEFPTVSMGLGPMDAIYQARFNRYLENRGIKDTSDQHVWAFLGDGEMDEPESRGLIQQAALNNLDNLTFVVNCNLQRLDGPVRGNTKIIQELESFFRGAGWSVIKVVWGREWDELLEKDQDGALVEIMNNTSDGDYQTFKANDGAYVREHFFGRDPRTAKLVENMTDEEIWKLPRGGHDYRKVYAAYKRALETKDRPTVILAHTIKGYGLGHNFEGRAATHEMKKLTLDDLKLFRDKQGIPITDEQLEKDPYLPPYYHPGEDAPEIKYMKERRAALGGYLPERRENYDPIQVPPLDKLRSVRKGSGKQQIATTMATVRTFKELMRDKGLADRLVPIIPDEARTFGLDSWFPTLKIYNPHGQNYVPVDHDLMLSYREAPEGQILHEGINEAGSVASFIAAGTSYATHGKAMIPLYIFYSMFGFQRTGDSIWAAADQMARGFLLGATAGRTTLTGEGLQHMDGHSPVLASTNEGVETYDPSFAYEIAHLVHRGIDRMYGPGKGEDVIYYITIYNEPTPQPAEPEGLDVEGLHKGIYLYSRGEGTGHEANILASGVGMQWALKAASILEADYGVRANIYSATSWVNLARDGAARNKAQLRNPGADAGEAFVTTQLKQTSGPYVAVSDFSTDLPNQIREWVPGDYTVLGADGFGFSDTRPAARRFFNIDAESIVVAVLNSLAREGKIDVSVAAQAAEKFKLDDPTSVSVDPNAPEE

SEQ ID NO: 31 - protein, 922 aa, Artificial Sequence
  N428A, K435A
MADQAKLGGKPSDDSNFAMIRDGVASYLNDSDPEETNEWMDSLDGLLQESSPERARYLMLRLLERASAKRVSLPPMTSTDYVNTIPTSMEPEFPGDEEMEKRYRRWIRWNAAIMVHRAQRPGIGVGGHISTYAGAAPLYEVGFNHFFRGKDHPGGGDQIFFQGHASPGMYARAFMEGRLSEDDLDGFRQEVSREQGGIPSYPHPHGMKDFWEFPTVSMGLGPMDAIYQARFNRYLENRGIKDTSDQHVWAFLGDGEMDEPESRGLIQQAALNNLDNLTFVVNCNLQRLDGPVRGNTKIIQELESFFRGAGWSVIKVVWGREWDELLEKDQDGALVEIMNNTSDGDYQTFKANDGAYVREHFFGRDPRTAKLVENMTDEEIWKLPRGGHDYRKVYAAYKRALETKDRPTVILAHTIKGYGLGHNFEGRAATHQMKALTLDDLKLFRDKQGIPITDEQLEKDPYLPPYYHPGEDAPEIKYMKERRAALGGYLPERRENYDPIQVPPLDKLRSVRKGSGKQQIATTMATVRTFKELMRDKGLADRLVPIIPDEARTFGLDSWFPTLKIYNPHGQNYVPVDHDLMLSYREAPEGQILHEGINEAGSVASFIAAGTSYATHGKAMIPLYIFYSMFGFQRTGDSIWAAADQMARGFLLGATAGRTTLTGEGLQHMDGHSPVLASTNEGVETYDPSFAYEIAHLVHRGIDRMYGPGKGEDVIYYITIYNEPTPQPAEPEGLDVEGLHKGIYLYSRGEGTGHEANILASGVGMQWALKAASILEADYGVRANIYSATSWVNLARDGAARNKAQLRNPGADAGEAFVTTQLKQTSGPYVAVSDFSTDLPNQIREWVPGDYTVLGADGFGFSDTRPAARRFFNIDAESIVVAVLNSLAREGKIDVSVAAQAAEKFKLDDPTSVSVDPNAPEE

SEQ ID NO: 32 - protein, 922 aa, Artificial Sequence
  Y418H, K435A
MADQAKLGGKPSDDSNFAMIRDGVASYLNDSDPEETNEWMDSLDGLLQESSPERARYLMLRLLERASAKRVSLPPMTSTDYVNTIPTSMEPEFPGDEEMEKRYRRWIRWNAAIMVHRAQRPGIGVGGHISTYAGAAPLYEVGFNHFFRGKDHPGGGDQIFFQGHASPGMYARAFMEGRLSEDDLDGFRQEVSREQGGIPSYPHPHGMKDFWEFPTVSMGLGPMDAIYQARFNRYLENRGIKDTSDQHVWAFLGDGEMDEPESRGLIQQAALNNLDNLTFVVNCNLQRLDGPVRGNTKIIQELESFFRGAGWSVIKVVWGREWDELLEKDQDGALVEIMNNTSDGDYQTFKANDGAYVREHFFGRDPRTAKLVENMTDEEIWKLPRGGHDYRKVYAAYKRALETKDRPTVILAHTIKGHGLGHNFEGRNATHQMKALTLDDLKLFRDKQGIPITDEQLEKDPYLPPYYHPGEDAPEIKYMKERRAALGGYLPERRENYDPIQVPPLDKLRSVRKGSGKQQIATTMATVRTFKELMRDKGLADRLVPIIPDEARTFGLDSWFPTLKIYNPHGQNYVPVDHDLMLSYREAPEGQILHEGINEAGSVASFIAAGTSYATHGKAMIPLYIFYSMFGFQRTGDSIWAAADQMARGFLLGATAGRTTLTGEGLQHMDGHSPVLASTNEGVETYDPSFAYEIAHLVHRGIDRMYGPGKGEDVIYYITIYNEPTPQPAEPEGLDVEGLHKGIYLYSRGEGTGHEANILASGVGMQWALKAASILEADYGVRANIYSATSWVNLARDGAARNKAQLRNPGADAGEAFVTTQLKQTSGPYVAVSDFSTDLPNQIREWVPGDYTVLGADGFGFSDTRPAARRFFNIDAESIVVAVLNSLAREGKIDVSVAAQAAEKFKLDDPTSVSVDPNAPEE

SEQ ID NO: 33 - protein, 922 aa, Artificial Sequence
  Y418H, Q432A
MADQAKLGGKPSDDSNFAMIRDGVASYLNDSDPEETNEWMDSLDGLLQESSPERARYLMLRLLERASAKRVSLPPMTSTDYVNTIPTSMEPEFPGDEEMEKRYRRWIRWNAAIMVHRAQRPGIGVGGHISTYAGAAPLYEVGFNHFFRGKDHPGGGDQIFFQGHASPGMYARAFMEGRLSEDDLDGFRQEVSREQGGIPSYPHPHGMKDFWEFPTVSMGLGPMDAIYQARFNRYLENRGIKDTSDQHVWAFLGDGEMDEPESRGLIQQAALNNLDNLTFVVNCNLQRLDGPVRGNTKIIQELESFFRGAGWSVIKVVWGREWDELLEKDQDGALVEIMNNTSDGDYQTFKANDGAYVREHFFGRDPRTAKLVENMTDEEIWKLPRGGHDYRKVYAAYKRALETKDRPTVILAHTIKGHGLGHNFEGRNATHAMKKLTLDDLKLFRDKQGIPITDEQLEKDPYLPPYYHPGEDAPEIKYMKERRAALGGYLPERRENYDPIQVPPLDKLRSVRKGSGKQQIATTMATVRTFKELMRDKGLADRLVPIIPDEARTFGLDSWFPTLKIYNPHGQNYVPVDHDLMLSYREAPEGQILHEGINEAGSVASFIAAGTSYATHGKAMIPLYIFYSMFGFQRTGDSIWAAADQMARGFLLGATAGRTTLTGEGLQHMDGHSPVLASTNEGVETYDPSFAYEIAHLVHRGIDRMYGPGKGEDVIYYITIYNEPTPQPAEPEGLDVEGLHKGIYLYSRGEGTGHEANILASGVGMQWALKAASILEADYGVRANIYSATSWVNLARDGAARNKAQLRNPGADAGEAFVTTQLKQTSGPYVAVSDFSTDLPNQIREWVPGDYTVLGADGFGFSDTRPAARRFFNIDAESIVVAVLNSLAREGKIDVSVAAQAAEKFKLDDPTSVSVDPNAPEE